European Patent Application EP 4 361 276 A1, published May 1, 2024. Title: RECOMBINANT MICROORGANISM WITH REGULATED EXPRESSION OF NADH:QUINONE OXIDOREDUCTASE AND METHOD FOR PRODUCING O-PHOSPHOSERINE, CYSTEINE, AND DERIVATIVES THEREOF USING THE SAME. Applicant: CJ CheilJedang Corporation. The sequence listing filed with the application follows.

SEQUENCE LISTING (39 sequences)

SEQ ID NO: 1 - DNA, 15655 bp, Artificial Sequence
  nuo operon
  misc_feature (1)..(630): nuoA promoter
  misc_feature (631)..(633): nuoA start codon
  misc_feature (1090)..(1092): nuoB start codon
  misc_feature (1846)..(1848): nuoC start codon
  misc_feature (3651)..(3653): nuoE start codon
  misc_feature (4148)..(4150): nuoF start codon
  misc_feature (5532)..(5534): nuoG start codon
  misc_feature (8261)..(8263): nuoH start codon
  misc_feature (9253)..(9255): nuoI start codon
  misc_feature (9807)..(9809): nuoJ start codon
  misc_feature (10358)..(10360): nuoK start codon
  misc_feature (10657)..(10659): nuoL start codon
  misc_feature (12662)..(12664): nuoM start codon
  misc_feature (14378)..(14380): nuoN start codon
tcgacggacgatagataattcctgagacaatagtgtaaaaaacgagccgctgggggtgttttaaaccccagcggcttttttttagtaaaaatccttcatcgcatagtgcagaacgtacaaaactgttcatttttcaaccaccagagattcacgtcccgaacgcacaaataatcgcctgaaaaaaatcacctgctacaatgatgttaaaaaatacgtaaatttgttgctgcgtttttgttatggaatgacaaaagcgtgtcacagatcaagaaaatactctcttttggggggaggaatcgacacaaattcctgtcaaaatagacccgtattttttccattgcttcacaacggacacgattcaacaacatctaattatcctggagtcgtcaaggatctggggtgaaagggcattaaatgctaatggtgttgatattatgtaaactaatgtgaagaaacttttgttaaagttgacaaaaggttatagaaaggagtaaaaaaccacatcaattagctgtataaaagaatttctacagtgattgtaaggttttttttattcctccccatgaatcgatgtggcgtccatctgccgtgaagagcagtgaatctggcgctacttttgatgagtaagcaatgagtatgtcaacatccactgaagtcatcgctcatcactgggcattcgctatctttcttatcgttgccattggcctgtgttgcctgatgctggtaggcggttggtttttaggcggtcgcgcacgcgcgaggtcgaaaaacgtgccgtttgaatccggtatcgactcggtcggctccgcccgcttacgcctgtccgccaagttttatctggtggccatgttcttcgttatcttcgacgttgaagcgctgtatctgttcgcatggtcaacctctatccgcgaaagcggctgggtaggctttgtggaagctgcaatttttatttttgtgttactggcaggtctggtttatctggtgcgtattggcgcgctggactggacgcccgcgcgttcacgccgcgagcgtatgaacccggaaacgaacagtatcgctaatcgtcaacgctaaccgcgaggcattaagatggattatacgctcacccgcatagatcccaacggtgagaacgaccgttaccccctgcaaaagcaggagatcgtaaccgaccctctggagcaagaagttaacaaaaacgtgtttatgggcaagctcaatgacatggttaactggggtcgtaaaaactcaatttggccgtataacttcggtctttcctgctgttacgttgagatggtgacttcgtttaccgcggtgcatgacgtggcgcgttttggcgcagaagtattgcgtgcttcgccgcgtcaggctgacctgatggtggttgcaggaacctgctttaccaaaatggcaccggttattcagcgtctgtatgaccagatgctggaaccaaaatgggttatctcaatgggtgcctgtgccaactctggtggtatgtacgatatttattccgttgtgcagggcgtcgataaattcatcccggttgatgtgtatatcccgggctgcccgccgcgtcctgaagcgtacatgcaggcactgatgctgttgcaggaatctatcggcaaagaacgtcgtccgctctcctgggtggttggcgatcagggcgtttatcgcgccaatatgcaatcagagcgcgaacgcaagcgcggtgaacgcattgccgtaactaacctgcgtacacctgacgagatttaatttgcgcctgtcggcaaagggatttttcttcgcttattcctaaatctatttcgcgaagcttactgcgccgacagtcaccacggaccatttgcaatggtgaacaatatgaccgacttaaccgcgcaagaacccgcctggcagacccgcgatcatcttgatgatccggtgattggcgaactgcgcaaccgttttgggccggatgcctttactgttcaggcgactcgcaccggggttcccgttgtgtggatcaagcgtgaacaattactggaagttggcgatttcttaaagaaactgccgaaaccttacgtcatgctgtttgacttacacggcatggacgaacgtctgcgcacacaccgcgaagggttacctgccgcggatttttccgttttctaccatctgatttctatcgatcgtaaccgcgacatcatgctgaaggtggcgctggcagaaaacgacctgcacgtaccgaccttcaccaaactgttcccgaacgctaactggtatgagcgtgaaacctgggatctgtttggcattactttcgacggtcacccgaacctgcgacgcatcatgatgccgcaaacctggaaaggtcacccgctgcgtaaagattatccggcgcgcgctaccgaattctcgccgtttgagctgaccaaagccaaacaggatctggagatggaagccctgaccttcaaaccggaagagtgggggatgaagcgcggcaccgaaaacgaggacttcatgttcctcaacctcggtccgaaccacccgtcggcgcacggggctttccgtatcgttttgcaactcgatggcgaagagattgtcgactgcgtaccagacatcggttaccaccaccgtggtgcggagaaaatgggcgaacgccagtcctggcacagctacattccgtatactgaccgtatcgaatacctcggcggctgcgttaacgaaatgccttacgtgctggcggtagagaaactggccgggatcaccgtgccggatcgcgttaacgtcattcgcgttatgctctccgaactgttccgcatcaacagtcacctgctgtatatctcgacctttattcaggacgtcggcgcaatgacgccagtgttcttcgcctttaccgatcgtcagaaaatttacgatctggtggaagcaatcactggtttccgtatgcacccggcgtggttccgtattggcggcgtagcgcacgacctgccgcgcggctgggatcgcctgctgcgtgagttcctcgactggatgccgaaacgtctggcgtcttacgagaaagcggcgctgcaaaacaccattctgaaaggtcgttcccagggcgttgccgcctatggcgcgaaagaggcgctggagtggggcaccactggcgcgggcctgcgtgctaccgggatcgacttcgacgtgcgtaaggcgcgtccttattctggctatgaaaacttcgactttgaaatcccggtgggtggtggcgtttctgactgctacacccgcgtaatgcttaaagtggaagagctgcgccagagtctgcgcattcttgagcagtgcctcaacaacatgccggaaggcccgttcaaagcggatcacccgctgaccacgccgccgccgaaagagcgcacgctgcaacatatcgaaaccctgatcacccacttcctgcaagtgtcgtggggtccggtgatgcctgccaatgaatctttccagatgattgaggcgaccaaagggatcaacagttactacctgaccagcgacggcagcaccatgagttaccgcacccgtgttcgtaccccgagctttgcgcatttgcagcaaattccggcggcgatccgcggcagcctggtgtctgacctgattgtttatctgggcagtatcgattttgttatgtcagatgtggaccgctaattatgcacgagaatcaacaaccacaaaccgaggcttttgagctgagtgcggcagagcgtgaagcgatcgagcacgagatgcaccactacgaagacccgcgtgcggcgtccattgaagcgctgaaaatcgttcagaagcagcgtggctgggtgccggatggtgcgatccacgcgatcgccgatgtgctgggtattccggcaagcgacgtcgaaggtgtggcaacgttctacagtcagatcttccgccagccggttggtcgccatgtgatccgttattgtgacagcgtggtctgtcatatcaacggttatcagggtattcaggcggcgctcgagaaaaagctgaacatcaaaccagggcaaacgacatttgatggccgctttacgctgctgccaacttgctgcctggggaactgtgataaagggccaaacatgatgatcgatgaggacactcacgcgcatctgaccccggaagcgatccctgaactgctggagcggtataaatgaaaaacattatccgtactcccgaaacgcatccgctgacctggcgtctgcgcgatgacaaacagccagtgtggctggacgaataccgcagcaaaaacggttacgaaggcgcgcgtaaggcgctgaccgggctgtctccggacgaaatcgttaatcaggtaaaagacgctggtctgaaagggcgcggcggcgcgggcttctcgactggcctgaaatggagcctgatgccgaaagacgaatccatgaacatccgttacctgctgtgtaatgccgatgaaatggagccgggcacctataaagaccgcctgttgatggagcaactgccgcacctgctggtggaaggtatgctcatctccgcgtttgcgctgaaagcttaccgtggctacatcttcctgcgtggcgaatatatcgaagcggcagttaatctgcgccgtgccattgccgaagccaccgaagcgggtctgcttggcaaaaacattatgggaacaggtttcgatttcgaactgttcgtccataccggggcagggcgctacatctgcggggaagaaacagcgttaatcaactccctggaaggacgtcgtgctaacccacgctcgaagccacccttcccggcaacctccggcgcatggggtaaaccgacctgtgtcaacaacgtcgaaaccctgtgtaacgttccggcgatcctcgctaacggcgtggagtggtatcagaacatctcgaaaagtaaagatgctggcaccaagctgatgggcttctccggtcgggtgaaaaatccgggactgtgggaactgccgttcggcaccaccgcacgcgagatcctcgaagattacgccggtggtatgcgtgatggtctgaaatttaaagcctggcagccaggcggcgcggggactgacttcctgaccgaagcgcaccttgatctgccgatggaattcgaaagtatcggtaaagcgggcagccgtctgggtacggcgctggcgatggcggttgaccatgagatcaacatggtgtcgctggtgcgtaacctggaagagtttttcgcccgtgagtcctgcggctggtgtacgccgtgccgcgacggtctgccgtggagcgtgaaaattctgcgtgcgctggagcgtggtgaaggtcagccgggcgatatcgaaacacttgagcaactgtgtcgattcttaggcccgggtaaaactttctgtgcccacgcacctggtgcagtggagccgttacagagcgccatcaaatatttccgcgaagaatttgaggcgggaatcaaacagccgttcagcaatacccatttgattaatgggattcagccgaacctgctgaaagagcgctggtaaccgaatttcgattaacgctcagtctctgactgagaaaactggaagcatgctaatggctacaattcatgtagacggcaaagaatacgaggtcaacggagcggacaacctgctggaagcttgtctgtctctgggccttgatattccttacttttgctggcatccggcgctgggaagtgtcggtgcttgccgccagtgtgcggtgaagcaataccaaaacgcggaagacacgcgtggtcgcctggtgatgtcctgtatgacaccggcttccgatggcacctttatttccattgacgacgaagaagcgaaacagttccgtgaaagcgtggtcgagtggttgatgaccaaccacccgcacgactgtccggtatgtgaagagggcggtaactgccatcttcaggatatgactgtgatgaccggacacagcttccgtcgctaccgtttcaccaaacgtacccaccgtaatcaggatttggggccattcatctctcacgaaatgaaccgctgcatcgcctgctaccgctgtgtgcgttactacaaagattacgctgacggtacagatctgggcgtttacggtgcgcacgacaacgtctacttcggtcgcccggaagacggcacgctggaaagcgaattttccggtaacctggtcgaaatttgcccgaccggcgtatttaccgacaaaacgcactccgagcgttacaaccgtaaatgggatatgcagtttgcgccgagcatctgccagcaatgttccatcggctgtaacatcagccccggtgaacgttacggcgaactgcgtcgtatcgaaaaccgttacaacggtacggtaaaccactacttcctctgcgaccgtggtcgtttcggttacggttacgtcaacctgaaggatcgtccgcgtcagccagtacagcgtcgtggcgatgatttcattaccctcaacgccgaacaggcaatgcagggcgcggcagatattctgcgtcagtcgaagaaagtgatcggtattggttctccgcgtgccagcgtggaaagcaactttgcgctgcgtgaactggtgggcgaagaaaacttctacaccggtatcgctcacggtgagcaggaacgtctgcaactggcgctgaaagtgctgcgtgaaggcggcatttatactccggctctgcgcgaaatcgaatcttacgatgcggtactggtgctgggcgaagacgttacccagaccggcgcgcgcgtcgcgctggcagtgcgtcaggctgtgaaaggtaaagcgcgcgaaatggcggcagcacagaaagtggctgactggcagattgcggcaatcctcaacatcggtcaacgtgcgaagcatccgctgtttgttaccaacgttgatgacacccgtctggatgatatcgcggcgtggacttaccgcgcaccggttgaagatcaggcgcgtttaggttttgccatcgcccatgcgctggataactctgcaccagcggttgacggtatcgaacctgagctgcaaagcaaaatcgacgtcatcgtgcaggcactggcaggtgcgaagaaaccgttgattatctccgggacgaacgccggtagcttagaggtgattcaggcggcggctaacgtcgcgaaagccctgaaaggtcgcggcgctgacgtcggtatcaccatgattgcccgttccgtcaacagcatggggctgggcattatgggtggcggttcgcttgaagaagcgttaaccgaactggaaaccggacgcgccgacgcggtggtggtgttggaaaacgatctgcatcgtcacgcttctgctatccgcgtgaatgctgcgctggctaaagcaccgctggtgatggtggttgatcatcaacgcacagcgattatggaaaacgcccatctggtactttctgctgccagctttgctgaaagcgacggtacggtgatcaacaacgaaggccgcgcccaacgtttcttccaggtttacgatcctgcttattacgacagcaaaactgtcatgctggaaagctggcgctggttacactcgctgcacagcaccctgctgagccgtgaagtggactggacgcagctcgaccatgtgattgacgctgttgtggcgaaaatcccggaactggcaggtatcaaagatgctgcgccggatgcgacattccgtattcgtgggcagaaactggcccgtgaaccgcaccgttacagcggtcgtaccgccatgcgcgccaatatcagcgttcatgagccgcgtcagccgcaggatattgacaccatgttcaccttctcgatggaaggtaacaaccagccgactgcgcaccgttcgcaagtgccgtttgcctgggcgccgggctggaactccccgcaggcgtggaacaaattccaggacgaagtgggcggcaaactgcgctttggcgatccgggcgtgcgtctgtttgaaaccagcgaaaatggtctggattacttcaccagcgtaccggcacgcttccagccgcaggacgggaaatggcgtatcgcgccgtattaccacctgtttggcagcgatgaattgtcacagcgtgctccggtcttccagagccgtatgccgcagccgtacatcaaactcaacccagcggatgccgcgaagttgggtgtgaacgcaggtacacgcgtctcctttagttacgatggcaacacggtcacgctgccggttgaaatcgccgaaggactgacggcagggcaggtgggcttgccgatgggtatgtccggcattgctccggtgctggctggcgcgcatcttgaggatctcaaggaggcacaacaatgagttggatatcaccggaactgattgagatcctgctgaccatcctcaaagcggtggtgatcctgctggtggttgtcacctgcggggcattcatgagctttggcgaacgtcgcctgctgggtctgttccagaaccgttacggacctaaccgtgttggctggggcggttcgctccagctggttgcggacatgatcaaaatgttctttaaagaagactggatcccgaaattctcggatcgcgtcatctttaccctggcaccgatgattgcctttacctcgctgctgctggcctttgcgattgtgccagtcagtccgggttgggtggttgccgacctgaacatcgggattttgttcttcctgatgatggcaggtctggcggtttacgcggtgctgtttgcgggctggtcaagtaacaacaaatactcgttgctgggtgcgatgcgtgcttctgcgcagaccctgagctacgaagtgttcctcgggctttccttgatgggcgtggtggcgcaggccggttcattcaacatgaccgacatcgtcaacagccaggcgcatgtgtggaacgttatcccgcaattctttggttttattacctttgccatcgcgggcgtggcggtatgtcaccgtcacccgtttgaccagccggaagccgagcaggaactggcggatggttaccacattgaatattccggtatgaagttcggtctgttcttcgtgggtgagtacatcgggattgtgaccatctctgcattgatggtgacgctgttcttcggtggctggcaaggcccgttgttaccgccattcatctggttcgcgctgaaaaccgcgttctttatgatgatgttcattttgattcgtgcgtcgttaccgcgtccgcgttatgaccaggtaatgtccttcggctggaaaatctgcctgccgctgacgctgatcaacttgctggtaacggcggctgtcattctctggcaggcgcaataaggggcaataagaccatgaccttaaaagaattgttagtaggtttcggcacccaggttcgtagtatctggatgatcggcctgcacgcgttcgccaaacgcgaaacgcgaatgtacccggaagagccggtctatctgccgccccgttatcgtggtcgtatcgttctgacccgcgacccggacggcgaagagcgttgcgtagcctgtaacctctgcgcggtagcctgcccggtcggctgtatctcgctgcaaaaagcagaaaccaaagacggtcgctggtacccggaatttttccgcatcaacttctcacgctgcattttctgtggtctgtgcgaagaagcctgtccgaccacggcgattcagttaaccccggatttcgaaatgggggaatacaagcgccaggatctggtttacgagaaagaggatctgctgatctccggtccgggcaaatacccggaatataacttctaccggatggcaggtatggcaatcgacggcaaagataagggcgaagcagagaacgaagccaagcctatcgacgtcaagagcctgttaccgtaaggagaggggcaatggagttcgctttttatatctgtggcctgatagccatacttgcgaccttgcgagtgatcacccataccaatccggtacacgcactgctgtacctgattatttcgctgctggcgatttccggggtgttcttctcactgggcgcttacttcgccggtgcgctggaaattatcgtctacgcgggtgccattatggtgctgttcgtgttcgtggtgatgatgctcaacctgggcggttcagaaatcgaacaggaacgccagtggctgaaaccgcaggtgtggattggtccggcaattttgtcggccatcatgctggtggtgattgtttacgccatcctcggtgttaacgatcagggtatcgacggtacgccaatcagtgctaaagcagtgggtattacgctgttcgggccttacgtactggcggtggaactggcttctatgctgctgctcgcaggtctggttgtggccttccacgtcggtcgtgaagagcgtgcgggtgaagtgctgagcaatcgtaaagacgacagcgcgaaaagaaaaacggaggagcacgcatgatccccttacaacatggactgatcctcgcggcaatcttattcgttcttggcttaaccggtctggttatccgtcgcaatctgctgtttatgttgattggtctggaaatcatgattaacgcctccgcgctggccttcgtggtcgccggaagctactggggccagaccgacggtcaggtgatgtacattctcgccatcagcctcgcggcggcagaagcgagtatcggccttgcgctgctgctgcaacttcaccgtcgtcgccagaacctgaacatcgattcagtaagtgagatgcgcggatgaacatgcttgccttaaccattattttgccattgattggcttcgtcctgctggcattctcccgtgggcgctggtctgaaaacgtctcggcgatcgtcggcgtaggctctgtgggcctggcggcgctggtaaccgcctttatcggcgttgatttcttcgctaacggcgagcagacatacagccagccgctgtggacgtggatgtcggtaggcgactttaacatcggttttaacctggtgctggacggcctgtcgctgaccatgctctcggtggtcactggtgtgggtttccttattcacatgtacgcctcctggtatatgcgcggtgaagagggctactctcgcttcttcgcttacaccaacctgttcatcgccagcatggtggttctggtgcttgccgacaacctgctgctgatgtacctcggctgggaaggcgtgggcctgtgctcctatctgctgatcgggttctattacaccgatccgaagaatggcgcagcggcaatgaaagcgttcgtcgtgacccgtgtgggtgacgtgttcctcgctttcgcactgttcattctttacaacgaactgggcaccctgaacttccgcgaaatggtggaactggcaccagcgcactttgctgacggcaataacatgctgatgtgggcgacgctgatgctgctgggcggtgcggtcggtaaatctgcgcagttgccgttgcagacatggcttgccgacgcgatggcgggcccgacgcctgtctccgcgctgatccacgccgcaaccatggtaaccgcgggtgtctacctgatcgcccgtacccacggcctgttcctgatgacgccggaagttctgcatctggtgggtattgtcggggcggttacgctgctgctggccggttttgccgcgctggtacagaccgacatcaaacgtgttctcgcttactctaccatgagccagattggctacatgttcctcgcgcttggcgtgcaggcatgggatgcggcgattttccacttgatgacccacgcgttctttaaagcgctgctgttcctggcatccggttccgtcattctggcctgccatcacgaacagaacatcttcaagatgggcggtctgcgtaaatctattccgctggtttatctctgcttcctggtgggcggcgcagcactgtcggcactaccgctggtcactgcgggcttcttcagtaaggatgagatcctcgcgggtgcgatggcgaatggtcatatcaatctgatggtggcaggtctggtcggtgcgtttatgacctcgctctacaccttccgtatgattttcatcgtcttccacggaaaagaacaaattcacgctcacgccgtgaaaggggtaactcacagcctgccgctgattgtgctgctgatcctttccaccttcgttggcgcactgattgtaccgccgctgcagggcgtgcttccgcaaacgacggaactggcgcacggcagcatgttgaccctggaaattacctctggcgtggtcgcggtggtcggcattctgctggcagcctggctgtggctgggtaaacgtactctggtgacctccatcgccaacagtgcgccgggccgtctgctgggcacctggtggtacaacgcctggggatttgactggctgtatgacaaagtgttcgtcaagccgttcctgggtattgcctggttgctgaaacgcgatccgctgaactcaatgatgaacatcccggctgtcctttcccgctttgcaggtaaaggtctgctgttaagtgagaacggctatctgcgctggtatgtggcatccatgagcatcggtgcggtcgtggtgctggcactgttgatggtactgcgttgagttaaggattgtgggattgcccctgggcatataagaacgtaggtcggataagccgccttcgcggtgcatccgacactacccccagtccgaagagaattttctgtcgtgagaattcgttgaaaatccggtcctgacgggacttttacaaggaataaagatcgccatgttactaccctggctaatattaattccctttattggcggcttcctgtgctggcagaccgaacgctttggcgtcaaggtgccacgctggatcgcgctgatcaccatgggattgacgctggcgctgtcgctgcaactgtggttgcagggcggttattcactgacgcaatccgccggaattccgcagtggcagtctgaattcgacatgccgtggatcccgcgttttggtatctctattcatctcgccattgacgggctgtcgctgctgatggtcgtgctgaccggtctgctcggtgtgctggcggtactatgttcgtggaaagagatcgaaaaatatcagggcttcttccacctcaacctgatgtggatcctgggcggcgttatcggcgtgttccttgccatcgacatgttcctgttcttcttcttctgggaaatgatgctggtgccgatgtacttcctgatcgcactgtgggggcataaagcctctgacggtaaaacgcgtatcacggcggcaaccaagttcttcatttacacccaggcgagtggcctggtgatgttgattgccatcctggcgctggtttttgttcactacaatgcgaccggcgtctggaccttcaactatgaagagctgctgaatacgccaatgtccagtggtgtggaatacctgttaatgctgggcttcttcatcgccttcgcagtcaaaatgccggtggttccgctgcatggctggctgccggatgcgcactcccaggctccgaccgccggttccgttgacctcgcggggatcttgctgaaaactgccgcttacggtttgctgcgtttctccctgccgctgttcccgaacgcgtcggcagagttcgcgccaattgctatgtggctgggtgttatcggcatcttctacggtgcgtggatggccttcgcccagaccgatatcaaacgtctgatcgcctacacctcggtttcccacatgggcttcgtgctgattgctatctacaccggcagccagttggcctaccagggcgcggtaatccagatgattgcgcacggtttgtcggcggcgggtctgtttattctttgtggtcagctttatgaacgtatccatacccgcgacatgcgcatgatgggcggtctgtggagcaagatgaaatggctgccagcactgtcgctgttctttgcggtggcaacgcttgggatgcctggcaccggtaacttcgtcggcgaatttatgattctgttcggcagcttccaggttgtaccggtgattaccgttatctctacctttgggctggtctttgcatctgtttattcgctggcgatgttacatcgcgcttacttcggtaaagcgaaaagccagattgccagccaggaactgccagggatgtcgctgcgtgagctgtttatgatcctgttgctggtggtgctgctggtactgctgggcttctatccgcagccgattctggatacctcgcactccgcgattggcaatatccagcagtggtttgttaattccgttactactacaaggccgtaaatcgccatgacaataactccacaaaacctgatcgcactgctaccgttgctgatcgtcggcttgacggtggtggttgtgatgctctccattgcgtggcgacgcaatcatttcctcaacgctacgctctcggttattgggcttaacgcggcgctggtttcgctctggtttgttggccaggcgggcgctatggacgttacgccgctgatgcgcgttgatggtttcgccatgctttacaccgggctggtattgttggcgagcctcgccacctgtactttcgcctacccgtggcttgaaggctataacgacaacaaggatgagttctacctgttggtgttaattgccgcgctgggcgggatcctgctggcgaatgccaaccatctggcgtctctgttcctcggtatcgaactgatctctttgccgctgtttggcctggtcggttacgctttccgccagaaacgttcactggaagccagtatcaaatacaccatcctttctgccgcagcgtcttctttcctgctgtttggtatggcgctggtgtatgcgcagtctggcgacctgtcgtttgtcgcgttgggtaaaaaccttggcgacggtatgctcaacgagccgctgttgctggcaggtttcggcctgatgattgttggcctcggcttcaaactctctctggtgccgttccacctgtggacgccagacgtataccagggcgcgcctgcgccggtttccactttcctggcgacggcgagcaaaatcgctatcttcggtgtggtgatgcgtctgttcctctacgcaccggtgggtgacagcgaagcgattcgcgtggtgctggcgattatcgcctttgcctccatcatcttcggtaacctgatggcgctgagccagaccaatatcaaacgtctgctcggttactcatctatctctcacctcggctatctgctggtagcgctgattgcgctgcaaaccggcgagatgtcgatggaagcggtaggggtttacctggccggttatctgttcagcagcctcggcgcgttcggcgtggtcagcctgatgtccagcccgtatcgtggcccggatgctgattccctgttctcttaccgcggtctgttctggcatcgtccgatcctcgcggcagtgatgacggtgatgatgctgtctctggccggtatcccgatgacgctgggctttatcggtaagttctacgtgctggcggtcggtgtccaggcacacttgtggtggctggtgggtgccgtggttgtcggttcggcaatcggcctctactactacctgcgcgtggcggtgagcctgtatcttcacgccccggaacaaccgggtcgcgatgcaccatcaaactggcagtacagcgcgggcggtatcgttgtgctgatctctgcactgttggtactggtgctgggtgtatggccacaaccgctgattagcattgtgcgtttggcaatgccgctgatgtaa

SEQ ID NO: 2 - protein, 322 aa, Artificial Sequence [sequence omitted]

SEQ ID NO: 3 - DNA, 969 bp, Artificial Sequence
  serB
atgcctaacattacctggtgcgacctgcctgaagatgtctctttatggccgggtctgcctctttcattaagtggtgatgaagtgatgccactggattaccacgcaggtcgtagcggctggctgctgtatggtcgtgggctggataaacaacgtctgacccaataccagagcaaactgggtgcggcgatggtgattgttgccgcctggtgcgtggaagattatcaggtgattcgtctggcaggttcactcaccgcacgggctacacgcctggcccacgaagcgcagctggatgtcgccccgctggggaaaatcccgcacctgcgcacgccgggtttgctggtgatggatatggactccaccgccatccagattgaatgtattgatgaaattgccaaactggccggaacgggcgagatggtggcggaagtaaccgaacgggcgatgcgcggcgaactcgattttaccgccagcctgcgcagccgtgtggcgacgctgaaaggcgctgacgccaatattctgcaacaggtgcgtgaaaatctgccgctgatgccaggcttaacgcaactggtgctcaagctggaaacgctgggctggaaagtggcgattgcctccggcggctttactttctttgctgaatacctgcgcgacaagctgcgcctgaccgccgtggtagccaatgaactggagatcatggacggtaaatttaccggcaatgtgatcggcgacatcgtagacgcgcagtacaaagcgaaaactctgactcgcctcgcgcaggagtatgaaatcccgctggcgcagaccgtggcgattggcgatggagccaatgacctgccgatgatcaaagcggcagggctggggattgcctaccatgccaagccaaaagtgaatgaaaaggcggaagtcaccatccgtcacgctgacctgatgggggtattctgcatcctctcaggcagcctgaatcagaagtaa

SEQ ID NO: 4 - protein, 405 aa, Artificial Sequence
  YhhS
MPEPVAEPALNGLRLNLRIVSIVMFNFASYLTIGLPLAVLPGYVHDVMGFSAFWAGLVISLQYFATLLSRPHAGRYADSLGPKKIVVFGLCGCFLSGLGYLTAGLTASLPVISLLLLCLGRVILGIGQSFAGTGSTLWGVGVVGSLHIGRVISWNGIVTYGAMAMGAPLGVVFYHWGGLQALALIIMGVALVAILLAIPRPTVKASKGKPLPFRAVLGRVWLYGMALALASAGFGVIATFITLFYDAKGWDGAAFALTLFSCAFVGTRLLFPNGINRIGGLNVAMICFSVEIIGLLLVGVATMPWMAKIGVLLAGAGFSLVFPALGVVAVKAVPQQNQGAALATYTVFMDLSLGVTGPLAGLVMSWAGVPVIYLAAAGLVAIALLLTWRLKKRPPEHVPEAASSS

SEQ ID NO: 5 - DNA, 1218 bp, Artificial Sequence
  yhhS
atgcccgaacccgtagccgaacccgcgctaaacggattgcgcctgaatttgcgcattgtctctatagtcatgtttaacttcgccagctacctcaccatcgggttgccgctcgctgtattaccgggctatgtccatgatgtgatgggctttagcgccttctgggcaggattggttatcagcctgcaatatttcgccaccttgctgagccgccctcatgccggacgttacgccgattcgctgggacccaaaaagattgtcgtcttcggtttatgcggctgctttttgagcggtctggggtatctgacggcaggattaaccgccagtctgcctgtcatcagcctgttattactttgcctggggcgcgtcatccttgggattgggcaaagttttgccggaacgggatcgaccctatggggcgttggcgtggttggctcgctgcatatcgggcgggtgatttcgtggaacggcattgtcacttacggggcgatggcgatgggtgcgccgttaggcgtcgtgttttatcactggggcggcttgcaggcgttagcgttaatcattatgggcgtggcgctggtggccattttgttggcgatcccgcgtccgacggtaaaagccagtaaaggcaaaccgctgccgtttcgcgcggtgcttgggcgcgtctggctgtacggtatggcgctggcactggcttccgccggatttggcgtcatcgccacctttatcacgctgttttatgacgctaaaggttgggacggtgcggctttcgcgctgacgctgtttagctgtgcgtttgtcggtacgcgtttgttattccctaacggcattaaccgtatcggtggcttaaacgtagcgatgatttgctttagcgttgagataatcggcctgctactggttggcgtggcgactatgccgtggatggcgaaaatcggcgtcttactggcgggggccgggttttcgctggtgttcccggcattgggtgtagtggcggtaaaagcggttccgcagcaaaatcagggggcggcgctggcaacttacaccgtatttatggatttatcgcttggcgtgactggaccactggctgggctggtgatgagctgggcgggcgtaccggtgatttatctggcggcggcgggactggtcgcaatcgcgttattactgacgtggcgattaaaaaaacggcctccggaacacgtccctgaggccgcctcatcatcttaa

SEQ ID NO: 6 - DNA, 35 bp, Artificial Sequence
  yhhS UP F
ctgcaggaattcgatgaaggtaaccactttttccg

SEQ ID NO: 7 - DNA, 35 bp, Artificial Sequence
  yhhS UP R
gagttgcagcaagcggaggatcaccacatttttac

SEQ ID NO: 8 - DNA, 35 bp, Artificial Sequence
  Ptrc F
aatgtggtgatcctccgcttgctgcaactctctca

SEQ ID NO: 9 - DNA, 35 bp, Artificial Sequence
  Ptrc R
tacgggttcgggcatgatagctctcctgtgtgaaa

SEQ ID NO: 10 - DNA, 35 bp, Artificial Sequence
  yhhS Down F
cacaggagagctatcatgcccgaacccgtagccga

SEQ ID NO: 11 - DNA, 35 bp, Artificial Sequence
  yhhS Down R
gtcgactagcgtgatagcggtttgcctttactggc

SEQ ID NO: 12 - DNA, 20 bp, Artificial Sequence
  yhhSP Conf F
agttgagcaaaaacgccagt

SEQ ID NO: 13 - DNA, 20 bp, Artificial Sequence
  yhhSP Conf R
gccataccgtacagccagac

SEQ ID NO: 14 - DNA, 35 bp, Artificial Sequence
  UP F1
ctgcaggaattcgatcaaccaccagagattcacgt

SEQ ID NO: 15 - DNA, 35 bp, Artificial Sequence
  UP R1
gcttcctgactccagtgcttactcatcaaaagtag

SEQ ID NO: 16 - DNA, 35 bp, Artificial Sequence
  Prmf F
tttgatgagtaagcactggagtcaggaagccgctt

SEQ ID NO: 17 - DNA, 35 bp, Artificial Sequence
  Prmf R
tgttgacatactcatgcctcgtttccctcatactg

SEQ ID NO: 18 - DNA, 35 bp, Artificial Sequence
  Down F1
tgagggaaacgaggcatgagtatgtcaacatccac

SEQ ID NO: 19 - DNA, 35 bp, Artificial Sequence
  Down R1
acggtgagaacgaccgttacatcacgctagtcgac

SEQ ID NO: 20 - DNA, 35 bp, Artificial Sequence
  UP R2
tcatttttcttcagctgcttactcatcaaaagtag

SEQ ID NO: 21 - DNA, 35 bp, Artificial Sequence
  Pidi F
tttgatgagtaagcagctgaagaaaaatgagcatg

SEQ ID NO: 22 - DNA, 39 bp, Artificial Sequence
  Pidi R
tgttgacatactcataatttctcacatgtaattctgatc

SEQ ID NO: 23 - DNA, 35 bp, Artificial Sequence
  Down F2
tacatgtgagaaattatgagtatgtcaacatccac

SEQ ID NO: 24 - DNA, 20 bp, Artificial Sequence
  NuoP Conf F
gagagctaccataatccgtg

SEQ ID NO: 25 - DNA, 20 bp, Artificial Sequence
  NuoP Conf R
catctcaacgtaacagcagg

SEQ ID NO: 26 - protein, 147 aa, Artificial Sequence
  NuoA
MSMSTSTEVIAHHWAFAIFLIVAIGLCCLMLVGGWFLGGRARARSKNVPFESGIDSVGSARLRLSAKFYLVAMFFVIFDVEALYLFAWSTSIRESGWVGFVEAAIFIFVLLAGLVYLVRIGALDWTPARSRRERMNPETNSIANRQR

SEQ ID NO: 27 - protein, 220 aa, Artificial Sequence
  NuoB
MDYTLTRIDPNGENDRYPLQKQEIVTDPLEQEVNKNVFMGKLNDMVNWGRKNSIWPYNFGLSCCYVEMVTSFTAVHDVARFGAEVLRASPRQADLMVVAGTCFTKMAPVIQRLYDQMLEPKWVISMGACANSGGMYDIYSVVQGVDKFIPVDVYIPGCPPRPEAYMQALMLLQESIGKERRPLSWVVGDQGVYRANMQSERERKRGERIAVTNLRTPDEI

SEQ ID NO: 28 - protein, 600 aa, Artificial Sequence
  NuoC
MVNNMTDLTAQEPAWQTRDHLDDPVIGELRNRFGPDAFTVQATRTGVPVVWIKREQLLEVGDFLKKLPKPYVMLFDLHGMDERLRTHREGLPAADFSVFYHLISIDRNRDIMLKVALAENDLHVPTFTKLFPNANWYERETWDLFGITFDGHPNLRRIMMPQTWKGHPLRKDYPARATEFSPFELTKAKQDLEMEALTFKPEEWGMKRGTENEDFMFLNLGPNHPSAHGAFRIVLQLDGEEIVDCVPDIGYHHRGAEKMGERQSWHSYIPYTDRIEYLGGCVNEMPYVLAVEKLAGITVPDRVNVIRVMLSELFRINSHLLYISTFIQDVGAMTPVFFAFTDRQKIYDLVEAITGFRMHPAWFRIGGVAHDLPRGWDRLLREFLDWMPKRLASYEKAALQNTILKGRSQGVAAYGAKEALEWGTTGAGLRATGIDFDVRKARPYSGYENFDFEIPVGGGVSDCYTRVMLKVEELRQSLRILEQCLNNMPEGPFKADHPLTTPPPKERTLQHIETLITHFLQVSWGPVMPANESFQMIEATKGINSYYLTSDGSTMSYRTRVRTPSFAHLQQIPAAIRGSLVSDLIVYLGSIDFVMSDVDR

SEQ ID NO: 29 - protein, 166 aa, Artificial Sequence
  NuoE
MHENQQPQTEAFELSAAEREAIEHEMHHYEDPRAASIEALKIVQKQRGWVPDGAIHAIADVLGIPASDVEGVATFYSQIFRQPVGRHVIRYCDSVVCHINGYQGIQAALEKKLNIKPGQTTFDGRFTLLPTCCLGNCDKGPNMMIDEDTHAHLTPEAIPELLERYK

SEQ ID NO: 30 - protein, 445 aa, Artificial Sequence
  NuoF
MKNIIRTPETHPLTWRLRDDKQPVWLDEYRSKNGYEGARKALTGLSPDEIVNQVKDAGLKGRGGAGFSTGLKWSLMPKDESMNIRYLLCNADEMEPGTYKDRLLMEQLPHLLVEGMLISAFALKAYRGYIFLRGEYIEAAVNLRRAIAEATEAGLLGKNIMGTGFDFELFVHTGAGRYICGEETALINSLEGRRANPRSKPPFPATSGAWGKPTCVNNVETLCNVPAILANGVEWYQNISKSKDAGTKLMGFSGRVKNPGLWELPFGTTAREILEDYAGGMRDGLKFKAWQPGGAGTDFLTEAHLDLPMEFESIGKAGSRLGTALAMAVDHEINMVSLVRNLEEFFARESCGWCTPCRDGLPWSVKILRALERGEGQPGDIETLEQLCRFLGPGKTFCAHAPGAVEPLQSAIKYFREEFEAGIKQPFSNTHLINGIQPNLLKERW

SEQ ID NO: 31 - protein, 910 aa, Artificial Sequence
  NuoG
MLMATIHVDGKEYEVNGADNLLEACLSLGLDIPYFCWHPALGSVGACRQCAVKQYQNAEDTRGRLVMSCMTPASDGTFISIDDEEAKQFRESVVEWLMTNHPHDCPVCEEGGNCHLQDMTVMTGHSFRRYRFTKRTHRNQDLGPFISHEMNRCIACYRCVRYYKDYADGTDLGVYGAHDNVYFGRPEDGTLESEFSGNLVEICPTGVFTDKTHSERYNRKWDMQFAPSICQQCSIGCNISPGERYGELRRIENRYNGTVNHYFLCDRGRFGYGYVNLKDRPRQPVQRRGDDFITLNAEQAMQGAADILRQSKKVIGIGSPRASVESNFALRELVGEENFYTGIAHGEQERLQLALKVLREGGIYTPALREIESYDAVLVLGEDVTQTGARVALAVRQAVKGKAREMAAAQKVADWQIAAILNIGQRAKHPLFVTNVDDTRLDDIAAWTYRAPVEDQARLGFAIAHALDNSAPAVDGIEPELQSKIDVIVQALAGAKKPLIISGTNAGSLEVIQAAANVAKALKGRGADVGITMIARSVNSMGLGIMGGGSLEEALTELETGRADAVVVLENDLHRHASAIRVNAALAKAPLVMVVDHQRTAIMENAHLVLSAASFAESDGTVINNEGRAQRFFQVYDPAYYDSKTVMLESWRWLHSLHSTLLSREVDWTQLDHVIDAVVAKIPELAGIKDAAPDATFRIRGQKLAREPHRYSGRTAMRANISVHEPRQPQDIDTMFTFSMEGNNQPTAHRSQVPFAWAPGWNSPQAWNKFQDEVGGKLRFGDPGVRLFETSENGLDYFTSVPARFQPQDGKWRIAPYYHLFGSDELSQRAPVFQSRMPQPYIKLNPADAAKLGVNAGTRVSFSYDGNTVTLPVEIAEGLTAGQVGLPMGMSGIAPVLAGAHLEDLKEAQQ

SEQ ID NO: 32 - protein, 325 aa, Artificial Sequence
  NuoH
MSWISPELIEILLTILKAVVILLVVVTCGAFMSFGERRLLGLFQNRYGPNRVGWGGSLQLVADMIKMFFKEDWIPKFSDRVIFTLAPMIAFTSLLLAFAIVPVSPGWVVADLNIGILFFLMMAGLAVYAVLFAGWSSNNKYSLLGAMRASAQTLSYEVFLGLSLMGVVAQAGSFNMTDIVNSQAHVWNVIPQFFGFITFAIAGVAVCHRHPFDQPEAEQELADGYHIEYSGMKFGLFFVGEYIGIVTISALMVTLFFGGWQGPLLPPFIWFALKTAFFMMMFILIRASLPRPRYDQVMSFGWKICLPLTLINLLVTAAVILWQAQ

SEQ ID NO: 33 - protein, 180 aa, Artificial Sequence
  NuoI
MTLKELLVGFGTQVRSIWMIGLHAFAKRETRMYPEEPVYLPPRYRGRIVLTRDPDGEERCVACNLCAVACPVGCISLQKAETKDGRWYPEFFRINFSRCIFCGLCEEACPTTAIQLTPDFEMGEYKRQDLVYEKEDLLISGPGKYPEYNFYRMAGMAIDGKDKGEAENEAKPIDVKSLLP

SEQ ID NO: 34 - protein, 184 aa, Artificial Sequence
  NuoJ
MEFAFYICGLIAILATLRVITHTNPVHALLYLIISLLAISGVFFSLGAYFAGALEIIVYAGAIMVLFVFVVMMLNLGGSEIEQERQWLKPQVWIGPAILSAIMLVVIVYAILGVNDQGIDGTPISAKAVGITLFGPYVLAVELASMLLLAGLVVAFHVGREERAGEVLSNRKDDSAKRKTEEHA

SEQ ID NO: 35 - protein, 100 aa, Artificial Sequence
  NuoK
MIPLQHGLILAAILFVLGLTGLVIRRNLLFMLIGLEIMINASALAFVVAGSYWGQTDGQVMYILAISLAAAEASIGLALLLQLHRRRQNLNIDSVSEMRG

SEQ ID NO: 36 - protein, 613 aa, Artificial Sequence
  NuoL
MNMLALTIILPLIGFVLLAFSRGRWSENVSAIVGVGSVGLAALVTAFIGVDFFANGEQTYSQPLWTWMSVGDFNIGFNLVLDGLSLTMLSVVTGVGFLIHMYASWYMRGEEGYSRFFAYTNLFIASMVVLVLADNLLLMYLGWEGVGLCSYLLIGFYYTDPKNGAAAMKAFVVTRVGDVFLAFALFILYNELGTLNFREMVELAPAHFADGNNMLMWATLMLLGGAVGKSAQLPLQTWLADAMAGPTPVSALIHAATMVTAGVYLIARTHGLFLMTPEVLHLVGIVGAVTLLLAGFAALVQTDIKRVLAYSTMSQIGYMFLALGVQAWDAAIFHLMTHAFFKALLFLASGSVILACHHEQNIFKMGGLRKSIPLVYLCFLVGGAALSALPLVTAGFFSKDEILAGAMANGHINLMVAGLVGAFMTSLYTFRMIFIVFHGKEQIHAHAVKGVTHSLPLIVLLILSTFVGALIVPPLQGVLPQTTELAHGSMLTLEITSGVVAVVGILLAAWLWLGKRTLVTSIANSAPGRLLGTWWYNAWGFDWLYDKVFVKPFLGIAWLLKRDPLNSMMNIPAVLSRFAGKGLLLSENGYLRWYVASMSIGAVVVLALLMVLR

SEQ ID NO: 37 - protein, 509 aa, Artificial Sequence
  NuoM
MLLPWLILIPFIGGFLCWQTERFGVKVPRWIALITMGLTLALSLQLWLQGGYSLTQSAGIPQWQSEFDMPWIPRFGISIHLAIDGLSLLMVVLTGLLGVLAVLCSWKEIEKYQGFFHLNLMWILGGVIGVFLAIDMFLFFFFWEMMLVPMYFLIALWGHKASDGKTRITAATKFFIYTQASGLVMLIAILALVFVHYNATGVWTFNYEELLNTPMSSGVEYLLMLGFFIAFAVKMPVVPLHGWLPDAHSQAPTAGSVDLAGILLKTAAYGLLRFSLPLFPNASAEFAPIAMWLGVIGIFYGAWMAFAQTDIKRLIAYTSVSHMGFVLIAIYTGSQLAYQGAVIQMIAHGLSAAGLFILCGQLYERIHTRDMRMMGGLWSKMKWLPALSLFFAVATLGMPGTGNFVGEFMILFGSFQVVPVITVISTFGLVFASVYSLAMLHRAYFGKAKSQIASQELPGMSLRELFMILLLVVLLVLLGFYPQPILDTSHSAIGNIQQWFVNSVTTTRP

SEQ ID NO: 38 - protein, 425 aa, Artificial Sequence
  NuoN
MDVTPLMRVDGFAMLYTGLVLLASLATCTFAYPWLEGYNDNKDEFYLLVLIAALGGILLANANHLASLFLGIELISLPLFGLVGYAFRQKRSLEASIKYTILSAAASSFLLFGMALVYAQSGDLSFVALGKNLGDGMLNEPLLLAGFGLMIVGLGFKLSLVPFHLWTPDVYQGAPAPVSTFLATASKIAIFGVVMRLFLYAPVGDSEAIRVVLAIIAFASIIFGNLMALSQTNIKRLLGYSSISHLGYLLVALIALQTGEMSMEAVGVYLAGYLFSSLGAFGVVSLMSSPYRGPDADSLFSYRGLFWHRPILAAVMTVMMLSLAGIPMTLGFIGKFYVLAVGVQAHLWWLVGAVVVGSAIGLYYYLRVAVSLYLHAPEQPGRDAPSNWQYSAGGIVVLISALLVLVLGVWPQPLISIVRLAMPLM

SEQ ID NO: 39 - DNA, 4695 bp, Artificial Sequence
  pSKH130
tcgaggccgcgattaaattccaacatggatgctgatttatatgggtataaatgggctcgcgataatgtcgggcaatcaggtgcgacaatctatcgattgtatgggaagcccgatgcgccagagttgtttctgaaacatggcaaaggtagcgttgccaatgatgttacagatgagatggtcagactaaactggctgacggaatttatgcctcttccgaccatcaagcattttatccgtactcctgatgatgcatggttactcaccactgcgatccccgggaaaacagcattccaggtattagaagaatatcctgattcaggtgaaaatattgttgatgcgctggcagtgttcctgcgccggttgcattcgattcctgtttgtaattgtccttttaacagcgatcgcgtatttcgtctcgctcaggcgcaatcacgaatgaataacggtttggttgatgcgagtgattttgatgacgagcgtaatggctggcctgttgaacaagtctggaaagaaatgcataagcttttgccattctcaccggattcagtcgtcactcatggtgatttctcacttgataaccttatttttgacgaggggaaattaataggttgtattgatgttggacgagtcggaatcgcagaccgataccaggatcttgccatcctatggaactgcctcggtgagttttctccttcattacagaaacggctttttcaaaaatatggtattgataatcctgatatgaataaattgcagtttcatttgatgctcgatgagtttttctaatcagaattggttaattggttgtaacactggcagagcattacgctgacttgacgggacggcggctttgttgaataaatcgaacttttgctgagttgaaggatcagatcacgcatcttcccgacaacgcagaccgttccgtggcaaagcaaaagttcaaaatcaccaactggtccacctacaacaaagctctcatcaaccgtggctccctcactttctggctggatgatggggcgattcaggcctggtatgagtcagcaacaccttcttcacgaggcagacctcagcgctcaaagatgcaggggtaaaagctaaccgcatctttaccgacaaggcatccggcagttcaacagatcgggaagggctggatttgctgaggatgaaggtggaggaaggtgatgtcattctggtgaagaagctcgaccgtcttggccgcgacaccgccgacatgatccaactgataaaagagtttgatgctcagggtgtagcggttcggtttattgacgacgggatcagtaccgacggtgatatggggcaaatggtggtcaccgcgcgtaatacgactcactatagggcgaattggagctccaccgcggtggcggccgctctagactttacggtatcgccgctcccgattcgcagcgcatcgccttctatcgccttcttgacgagttcttctgagcgggactctggggttcgctagaggatcgatcctttttaacccatcacatatacctgccgttcactattatttagtgaaatgagatattatgatattttctgaattgtgattaaaaaggcaactttatgcccatgcaacagaaactataaaaaatacagagaatgaaaagaaacagatagattttttagttctttaggcccgtagtctgcaaatccttttatgattttctatcaaacaaaagaggaaaatagaccagttgcaatccaaacgagagtctaatagaatgaggtcgaaaagtaaatcgcgcgggtttgttactgataaagcaggcaagacctaaaatgtgtaaagggcaaagtgtatactttggcgtcaccccttacatattttaggtctttttttattgtgcgtaactaacttgccatcttcaaacaggagggctggaagaagcagaccgctaacacagtacataaaaaaggagacatgaacgatgaacatcaaaaagtttgcaaaacaagcaacagtattaacctttactaccgcactgctggcaggaggcgcaactcaagcgtttgcgaaagaaacgaaccaaaagccatataaggaaacatacggcatttcccatattacacgccatgatatgctgcaaatccctgaacagcaaaaaaatgaaaaatatcaagttcctgaattcgattcgtccacaattaaaaatatctcttctgcaaaaggcctggacgtttgggacagctggccattacaaaacgctgacggcactgtcgcaaactatcacggctaccacatcgtctttgcattagccggagatcctaaaaatgcggatgacacatcgatttacatgttctatcaaaaagtcggcgaaacttctattgacagctggaaaaacgctggccgcgtctttaaagacagcgacaaattcgatgcaaatgattctatcctaaaagaccaaacacaagaatggtcaggttcagccacatttacatctgacggaaaaatccgtttattctacactgatttctccggtaaacattacggcaaacaaacactgacaactgcacaagttaacgtatcagcatcagacagctctttgaacatcaacggtgtagaggattataaatcaatctttgacggtgacggaaaaacgtatcaaaatgtacagcagttcatcgatgaaggcaactacagctcaggcgacaaccatacgctgagagatcctcactacgtagaagataaaggccacaaatacttagtatttgaagcaaacactggaactgaagatggctaccaaggcgaagaatctttatttaacaaagcatactatggcaaaagcacatcattcttccgtcaagaaagtcaaaaacttctgcaaagcgataaaaaacgcacggctgagttagcaaacggcgctctcggtatgattgagctaaacgatgattacacactgaaaaaagtgatgaaaccgctgattgcatctaacacagtaacagatgaaattgaacgcgcgaacgtctttaaaatgaacggcaaatggtacctgttcactgactcccgcggatcaaaaatgacgattgacggcattacgtctaacgatatttacatgcttggttatgtttctaattctttaactggcccatacaagccgctgaacaaaactggccttgtgttaaaaatggatcttgatcctaacgatgtaacctttacttactcacacttcgctgtacctcaagcgaaaggaaacaatgtcgtgattacaagctatatgacaaacagaggattctacgcagacaaacaatcaacgtttgcgccaagcttcctgctgaacatcaaaggcaagaaaacatctgttgtcaaagacagcatccttgaacaaggacaattaacagttaacaaataaaaacgcaaaagaaaatgccgatgggtaccgagcgaaatgaccgaccaagcgacgcccaacctgccatcggatcccccgggctgcaggaattcgatatcacgctagtcgacctagctagcatatggggagatctactagtaaagcatgccaattggtattctatagtgtcacctaaatcgtatgtgtatgatacataaggttatgtattaattgtagccgcgttctaacgacaatatgtacaagcctaattgtgtagcatctggcttactgaagcagaccctatcatctctctcgtaaactgccgtcagagtcggtttggttggacgaaccttctgagtttctggtaacgccgtcccgcacccggaaatggtcagcgaaccaatcagcagggtcatcgctagcccatggctaattcccatgtcagccgttaagtgttcctgtgtcactcaaaattgctttgagaggctctaagggcttctcagtgcgttacatccctggcttgttgtccacaaccgttaaaccttaaaagctttaaaagccttatatattcttttttttcttataaaacttaaaaccttagaggctatttaagttgctgatttatattaattttattgttcaaacatgagagcttagtacgtgaaacatgagagcttagtacgttagccatgagagcttagtacgttagccatgagggtttagttcgttaaacatgagagcttagtacgttaaacatgagagcttagtacgtgaaacatgagagcttagtacgtactatcaacaggttgaactgctgatcttcagatcctctacgccggacgcatcgtggccggatcttgcggccgcaaaaattaaaaatgaagttttaaatcaatctaaagtatatatgagtaaacttggtctgacagttaccaatgcttaatcagtgaggcaccaataactgccttaaaaaaactagcgctgaggtctgcctcgtgaagaaggtgttgctgactcataccaggcctgaatcgccccatcatccagccagaaagtgagggagccacggttgatgagagctttgttgtaggtggaccagttggtgattttgaacttttgctttgccacggaacggtctgcgttgtcgggaagatgcgtgatctgatccttcaactcagcaaaagttcgatttattcaacaaagccacgttgtgtctcaaaatctctgatgttacattgcacaagataaaaatatatcatcatgaacaataaaactgtctgcttacataaacagtaatacaaggggtgttatgagccatattcaacgggaaacgtcttgc